European Patent Application EP 4 296 274 A1, published December 27, 2023. Title: PEPTIDES FOR INTRACELLULAR DELIVERY. Applicant: UNIVERSIDADE DE SANTIAGO DE COMPOSTELA. The sequence listing filed with the application follows.

SEQUENCE LISTING (64 sequences)

SEQ ID NO: 1 - protein, 7 aa, Artificial Sequence
  MOD_RES 1: ACETYLATION
  Cationic peptide 7.3(L-H)
  MOD_RES 2..2: Native lysine or modified lysine, wherein the modified lysine is a lysine forming an amide bond with a linker through the e-amino group.
  MOD_RES 5..5: Native lysine or modified lysine, wherein the modified lysine is a lysine forming an amide bond with a linker through the e-amino group.
  MOD_RES 6..6: Native lysine or modified lysine, wherein the modified lysine is a lysine forming an amide bond with a linker through the e-amino group.
  MOD_RES 7: AMIDATION
RKHRKKH

SEQ ID NO: 2 - protein, 7 aa, Artificial Sequence
  MOD_RES 1: ACETYLATION
  Cationic peptide V1-7.3(Leu-His)
  MOD_RES 3..3: Native lysine or modified lysine, wherein the modified lysine is a lysine forming an amide bond with a linker through the e-amino group.
  MOD_RES 4..4: Native lysine or modified lysine, wherein the modified lysine is a lysine forming an amide bond with a linker through the e-amino group.
  MOD_RES 5..5: Native lysine or modified lysine, wherein the modified lysine is a lysine forming an amide bond with a linker through the e-amino group.
  MOD_RES 7: AMIDATION
RHKKKHR

SEQ ID NO: 3 - protein, 7 aa, Artificial Sequence
  MOD_RES 1: ACETYLATION
  Cationic peptide V2-7.3(Leu-His)
  MOD_RES 2..2: Native lysine or modified lysine, wherein the modified lysine is a lysine forming an amide bond with a linker through the e-amino group.
  MOD_RES 5..5: Native lysine or modified lysine, wherein the modified lysine is a lysine forming an amide bond with a linker through the e-amino group.
  MOD_RES 6..6: Native lysine or modified lysine, wherein the modified lysine is a lysine forming an amide bond with a linker through the e-amino group.
  MOD_RES 7: AMIDATION
RKHHKKR

SEQ ID NO: 4 - protein, 7 aa, Artificial Sequence
  Peptide
  VARIANT 2..2
  VARIANT 3..3
  VARIANT 6..6
  VARIANT 7..7
RXXRRXX

SEQ ID NO: 5 - protein, 9 aa, Artificial Sequence
  Peptide
  VARIANT 2..2
  VARIANT 3..3
  VARIANT 6..6
  VARIANT 7..7
  VARIANT 9..9
RXXRRXXRX

SEQ ID NO: 6 - protein, 13 aa, Artificial Sequence
  Peptide
  VARIANT 3..3
  VARIANT 4..4
  VARIANT 6..6
  VARIANT 7..7
  VARIANT 10..10
  VARIANT 11..11
  VARIANT 13..13
RRXXRXXRRXXRX

SEQ ID NO: 7 - protein, 17 aa, Artificial Sequence
  Peptide
  VARIANT 3..3
  VARIANT 4..4
  VARIANT 6..6
  VARIANT 7..7
  VARIANT 10..10
  VARIANT 11..11
  VARIANT 13..13
  VARIANT 14..14
  VARIANT 17..17
RRXXRXXRRXXRXXRRX

SEQ ID NO: 8 - protein, 21 aa, Artificial Sequence
  Peptide
  VARIANT 3..3
  VARIANT 4..4
  VARIANT 6..6
  VARIANT 7..7
  VARIANT 10..10
  VARIANT 11..11
  VARIANT 13..13
  VARIANT 14..14
  VARIANT 17..17
RRXXRXXRRXXRXXRRXRRLL

SEQ ID NO: 9 - protein, 4 aa, Artificial Sequence
  Peptide
  VARIANT 2..2
  VARIANT 3..3
RXXR

SEQ ID NO: 10 - protein, 13 aa, Artificial Sequence
  Peptide
  VARIANT 2..2
  VARIANT 3..3
  VARIANT 4..4
  VARIANT 6..6
  VARIANT 7..7
  VARIANT 10..10
  VARIANT 11..11
  VARIANT 13..13
RXXXRXXRRXXRX

SEQ ID NO: 11 - protein, 7 aa, Artificial Sequence
  MOD_RES 1: ACETYLATION
  Cationic peptide 7.3
  MOD_RES 2..2: Native lysine or modified lysine, wherein the modified lysine is a lysine forming an amide bond with a linker through the e-amino group.
  MOD_RES 5..5: Native lysine or modified lysine, wherein the modified lysine is a lysine forming an amide bond with a linker through the e-amino group.
  MOD_RES 6..6: Native lysine or modified lysine, wherein the modified lysine is a lysine forming an amide bond with a linker through the e-amino group.
  MOD_RES 7: AMIDATION
RKLRKKL

SEQ ID NO: 12 - protein, 7 aa, Artificial Sequence
  MOD_RES 1: ACETYLATION
  Cationic peptide 7.3(Leu-Arg)
  MOD_RES 2..2: Native lysine or modified lysine, wherein the modified lysine is a lysine forming an amide bond with a linker through the e-amino group.
  MOD_RES 5..5: Native lysine or modified lysine, wherein the modified lysine is a lysine forming an amide bond with a linker through the e-amino group.
  MOD_RES 6..6: Native lysine or modified lysine, wherein the modified lysine is a lysine forming an amide bond with a linker through the e-amino group.
  MOD_RES 7: AMIDATION
RKRRKKR

SEQ ID NO: 13 - protein, 9 aa, Artificial Sequence
  MOD_RES 1: ACETYLATION
  Cationic peptide 9.3
  MOD_RES 2..2: Native lysine or modified lysine, wherein the modified lysine is a lysine forming an amide bond with a linker through the e-amino group.
  MOD_RES 6..6: Native lysine or modified lysine, wherein the modified lysine is a lysine forming an amide bond with a linker through the e-amino group.
  MOD_RES 9..9: Native lysine or modified lysine, wherein the modified lysine is a lysine forming an amide bond with a linker through the e-amino group.
  MOD_RES 9: AMIDATION
RKLRRKLRK

SEQ ID NO: 14 - protein, 13 aa, Artificial Sequence
  MOD_RES 1: ACETYLATION
  Cationic peptide 13.3
  MOD_RES 4..4: Native lysine or modified lysine, wherein the modified lysine is a lysine forming an amide bond with a linker through the e-amino group.
  MOD_RES 7..7: Native lysine or modified lysine, wherein the modified lysine is a lysine forming an amide bond with a linker through the e-amino group.
  MOD_RES 11..11: Native lysine or modified lysine, wherein the modified lysine is a lysine forming an amide bond with a linker through the e-amino group.
  MOD_RES 13: AMIDATION
RRLKRLKRRLKRL

SEQ ID NO: 15 - protein, 13 aa, Artificial Sequence
  MOD_RES 1: ACETYLATION
  Cationic peptide 13.3(2+1)
  MOD_RES 4..4: Native lysine or modified lysine, wherein the modified lysine is a lysine forming an amide bond with a linker through the e-amino group.
  MOD_RES 6..6: Native lysine or modified lysine, wherein the modified lysine is a lysine forming an amide bond with a linker through the e-amino group.
  MOD_RES 11..11: Native lysine or modified lysine, wherein the modified lysine is a lysine forming an amide bond with a linker through the e-amino group.
  MOD_RES 13: AMIDATION
RRLKRKLRRLKRL

SEQ ID NO: 16 - protein, 13 aa, Artificial Sequence
  MOD_RES 1: ACETYLATION
  Cationic peptide 13.3(3b)
  MOD_RES 3..3: Native lysine or modified lysine, wherein the modified lysine is a lysine forming an amide bond with a linker through the e-amino group.
  MOD_RES 4..4: Native lysine or modified lysine, wherein the modified lysine is a lysine forming an amide bond with a linker through the e-amino group.
  MOD_RES 6..6: Native lysine or modified lysine, wherein the modified lysine is a lysine forming an amide bond with a linker through the e-amino group.
  MOD_RES 13: AMIDATION
RRKKRKLRRLLRL

SEQ ID NO: 17 - protein, 13 aa, Artificial Sequence
  MOD_RES 1: ACETYLATION
  Cationic peptide 13.3(Leu-His)
  MOD_RES 4..4: Native lysine or modified lysine, wherein the modified lysine is a lysine forming an amide bond with a linker through the e-amino group.
  MOD_RES 7..7: Native lysine or modified lysine, wherein the modified lysine is a lysine forming an amide bond with a linker through the e-amino group.
  MOD_RES 11..11: Native lysine or modified lysine, wherein the modified lysine is a lysine forming an amide bond with a linker through the e-amino group.
  MOD_RES 13: AMIDATION
RRHKRLKRRLKRL

SEQ ID NO: 18 - protein, 13 aa, Artificial Sequence
  MOD_RES 1: ACETYLATION
  Cationic peptide 13.3(R-H)
  MOD_RES 4..4: Native lysine or modified lysine, wherein the modified lysine is a lysine forming an amide bond with a linker through the e-amino group.
  MOD_RES 7..7: Native lysine or modified lysine, wherein the modified lysine is a lysine forming an amide bond with a linker through the e-amino group.
  MOD_RES 11..11: Native lysine or modified lysine, wherein the modified lysine is a lysine forming an amide bond with a linker through the e-amino group.
  MOD_RES 13: AMIDATION
RHLKRLKRRLKRL

SEQ ID NO: 19 - protein, 13 aa, Artificial Sequence
  MOD_RES 1: ACETYLATION
  Cationic peptide 13.3(3His)
  MOD_RES 4..4: Native lysine or modified lysine, wherein the modified lysine is a lysine forming an amide bond with a linker through the e-amino group.
  MOD_RES 7..7: Native lysine or modified lysine, wherein the modified lysine is a lysine forming an amide bond with a linker through the e-amino group.
  MOD_RES 11..11: Native lysine or modified lysine, wherein the modified lysine is a lysine forming an amide bond with a linker through the e-amino group.
  MOD_RES 13: AMIDATION
RHLKRHKRRLKRH

SEQ ID NO: 20 - skipped

SEQ ID NO: 21 - protein, 17 aa, Artificial Sequence
  MOD_RES 1: ACETYLATION
  Cationic peptide 17.3
  MOD_RES 4..4: Native lysine or modified lysine, wherein the modified lysine is a lysine forming an amide bond with a linker through the e-amino group.
  MOD_RES 11..11: Native lysine or modified lysine, wherein the modified lysine is a lysine forming an amide bond with a linker through the e-amino group.
  MOD_RES 14..14: Native lysine or modified lysine, wherein the modified lysine is a lysine forming an amide bond with a linker through the e-amino group.
  MOD_RES 17: AMIDATION
RRLKRLLRRLKRLKRRL

SEQ ID NO: 22 - skipped

SEQ ID NO: 23 - protein, 21 aa, Artificial Sequence
  MOD_RES 1: ACETYLATION
  Cationic peptide 21.3
  MOD_RES 4..4: Native lysine or modified lysine, wherein the modified lysine is a lysine forming an amide bond with a linker through the e-amino group.
  MOD_RES 11..11: Native lysine or modified lysine, wherein the modified lysine is a lysine forming an amide bond with a linker through the e-amino group.
  MOD_RES 14..14: Native lysine or modified lysine, wherein the modified lysine is a lysine forming an amide bond with a linker through the e-amino group.
  MOD_RES 21: AMIDATION
RRLKRLLRRLKRLKRRLRRLL

SEQ ID NO: 24-25 - skipped (2 entries)

SEQ ID NO: 26 - protein, 7 aa, Artificial Sequence
  MOD_RES 1..1: ACETYLATION
  Cationic peptide 7.2
  MOD_RES 2..2: Native lysine or modified lysine, wherein the modified lysine is a lysine forming an amide bond with a linker through the e-amino group.
  MOD_RES 6..6: Native lysine or modified lysine, wherein the modified lysine is a lysine forming an amide bond with a linker through the e-amino group.
  MOD_RES 7..7: AMIDATION
RKLRRKL

SEQ ID NO: 27 - RNA, 3822 nt, Artificial Sequence
  Prefusion stabilized SARS-CoV-2 Spike protein mRNA open reading frame sequence
auguucguguuucuggugcugcugccucugguguccagccagugugugaaccugaccacaagaacccagcugccuccagccuacaccaacagcuuuaccagaggcguguacuaccccgacaagguguucagauccagcgugcugcacucuacccaggaccuguuccugccuuucuucagcaacgugaccugguuccacgccauccacguguccggcaccaauggcaccaagagauucgacaaccccgugcugcccuucaacgacgggguguacuuugccagcaccgagaaguccaacaucaucagaggcuggaucuucggcaccacacuggacagcaagacccagagccugcugaucgugaacaacgccaccaacguggucaucaaagugugcgaguuccaguucugcaacgaccccuuccugggcgucuacuaucacaagaacaacaagagcuggauggaaagcgaguuccggguguacagcagcgccaacaacugcaccuucgaguacgugucccagccuuuccugauggaccuggaaggcaagcagggcaacuucaagaaccugcgcgaguucguguucaagaacaucgacggcuacuucaagaucuacagcaagcacaccccuaucaaccucgugcgggaucugccucagggcuucucugcucuggaaccccugguggaucugcccaucggcaucaacaucacccgguuucagacacugcuggcccugcacagaagcuaccugacaccuggcgauagcagcagcggauggacagcuggugccgccgcuuacuaugugggcuaccugcagccuagaaccuuucugcugaaguacaacgagaacggcaccaucaccgacgccguggauugugcucuggauccucugagcgagacaaagugcacccugaaguccuucaccguggaaaagggcaucuaccagaccagcaacuuccgggugcagcccaccgaauccaucgugcgguuccccaauaucaccaaucugugccccuucggcgagguguucaaugccaccagauucgccucuguguacgccuggaaccggaagcggaucagcaauugcguggccgacuacuccgugcuguacaacuccgccagcuucagcaccuucaagugcuacggcguguccccuaccaagcugaacgaccugugcuucacaaacguguacgccgacagcuucgugauccggggagaugaagugcggcagauugccccuggacagacaggcaagaucgccgacuacaacuacaagcugcccgacgacuucaccggcugugugauugccuggaacagcaacaaccuggacuccaaagucggcggcaacuacaauuaccuguaccggcuguuccggaaguccaaucugaagcccuucgagcgggacaucuccaccgagaucuaucaggccggcagcaccccuuguaacggcguggaaggcuucaacugcuacuucccacugcaguccuacggcuuucagcccacaaauggcgugggcuaucagcccuacagagugguggugcugagcuucgaacugcugcaugccccugccacagugugcggcccuaagaaaagcaccaaucucgugaagaacaaaugcgugaacuucaacuucaacggccugaccggcaccggcgugcugacagagagcaacaagaaguuccugccauuccagcaguuuggccgggauaucgccgauaccacagacgccguuagagauccccagacacuggaaauccuggacaucaccccuugcagcuucggcggagugucugugaucaccccuggcaccaacaccagcaaucagguggcagugcuguaccaggacgugaacuguaccgaagugcccguggccauucacgccgaucagcugacaccuacauggcggguguacuccaccggcagcaauguguuucagaccagagccggcugucugaucggagccgagcacgugaacaauagcuacgagugcgacauccccaucggcgcuggcaucugugccagcuaccagacacagacaaacagccccggcagcgccagcucuguggccagccagagcaucauugccuacacaaugucucugggcgccgagaacagcguggccuacuccaacaacucuaucgcuauccccaccaacuucaccaucagcgugaccacagagauccugccuguguccaugaccaagaccagcguggacugcaccauguacaucugcggcgauuccaccgagugcuccaaccugcugcugcaguacggcagcuucugcacccagcugaauagagcccugacagggaucgccguggaacaggacaagaacacccaagagguguucgcccaagugaagcagaucuacaagaccccuccuaucaaggacuucggcggcuucaauuucagccagauucugcccgauccuagcaagcccagcaagcggagcuucaucgaggaccugcuguucaacaaagugacacuggccgacgccggcuucaucaagcaguauggcgauugucugggcgacauugccgccagggaucugauuugcgcccagaaguuuaacggacugacagugcugccuccucugcugaccgaugagaugaucgcccaguacacaucugcccugcuggccggcacaaucacaagcggcuggacauuuggagcuggcgccgcucugcagauccccuuugcuaugcagauggccuaccgguucaacggcaucggagugacccagaaugugcuguacgagaaccagaagcugaucgccaaccaguucaacagcgccaucggcaagauccaggacagccugagcagcacagcaagcgcccugggaaagcugcaggacguggucaaccagaaugcccaggcacugaacacccuggucaagcagcuguccuccaacuucggcgccaucagcucugugcugaacgauauccugagcagacuggacccgccggaagccgaggugcagaucgacagacugaucaccggaaggcugcagucccugcagaccuacguuacccagcagcugaucagagccgccgagauuagagccucugccaaucuggccgccaccaagaugucugagugugugcugggccagagcaagagaguggacuuuugcggcaagggcuaccaccugaugagcuucccucagucugccccucacggcgugguguuucugcacgugacauacgugcccgcucaagagaagaauuucaccaccgcuccagccaucugccacgacggcaaagcccacuuuccuagagaaggcguguucguguccaacggcacccauugguucgugacccagcggaacuucuacgagccccagaucaucaccaccgacaacaccuucgugucuggcaacugcgacgucgugaucggcauugugaacaauaccguguacgacccucugcagcccgagcuggacagcuucaaagaggaacuggauaaguacuuuaagaaccacacaagccccgacguggaccugggcgauaucagcggaaucaaugccagcgucgugaacauccagaaagagaucgaccggcugaacgagguggccaagaaucugaacgagagccugaucgaccugcaagaacuggggaaguacgagcaguacaucaaguggcccugguacaucuggcugggcuuuaucgccggacugauugccaucgugauggucacaaucaugcuguguugcaugaccagcugcuguagcugccugaagggcuguuguagcuguggcagcugcugcaaguucgacgaggacgauucugagcccgugcugaagggcgugaaacugcacuacaccuga

SEQ ID NO: 28-30 - skipped (3 entries)

SEQ ID NO: 31 - protein, 9 aa, Artificial Sequence
  MOD_RES 1..1: ACETYLATION
  Cationic peptide 9.2
  MOD_RES 2..2: Native lysine or modified lysine, wherein the modified lysine is a lysine forming an amide bond with a linker through the e-amino group.
  MOD_RES 9..9: AMIDATION
  MOD_RES 9..9: Native lysine or modified lysine, wherein the modified lysine is a lysine forming an amide bond with a linker through the e-amino group.
RKLRRLLRK

SEQ ID NO: 32-33 - skipped (2 entries)

SEQ ID NO: 34 - protein, 13 aa, Artificial Sequence
  MOD_RES 1..1: ACETYLATION
  Cationic peptide 13.2
  MOD_RES 4..4: Native lysine or modified lysine, wherein the modified lysine is a lysine forming an amide bond with a linker through the e-amino group.
  MOD_RES 11..11: Native lysine or modified lysine, wherein the modified lysine is a lysine forming an amide bond with a linker through the e-amino group.
  MOD_RES 13..13: AMIDATION
RRLKRLLRRLKRL

SEQ ID NO: 35-48 - skipped (14 entries)

SEQ ID NO: 49 - protein, 7 aa, Artificial Sequence
  MOD_RES 1..1: ACETYLATION
  Cationic peptide
  MOD_RES 2..2: Native lysine or modified lysine, wherein the modified lysine is a lysine forming an amide bond with a linker through the e-amino group
  MOD_RES 4..4: Native lysine or modified lysine, wherein the modified lysine is a lysine forming an amide bond with a linker through the e-amino group.
  MOD_RES 6..6: Native lysine or modified lysine, wherein the modified lysine is a lysine forming an amide bond with a linker through the e-amino group.
  MOD_RES 7..7: AMIDATION
RKHKHKR

SEQ ID NO: 50-51 - skipped (2 entries)

SEQ ID NO: 52 - protein, 7 aa, Artificial Sequence
  MOD_RES 1..1: ACETYLATION
  Cationic peptide 7.3(L-H)(K-O)
  MOD_RES 2..2: Native ornithine or modified ornithine wherein the modified ornithine is an ornithine forming an amide bond with a linker through the d-amino group
  MOD_RES 5: Native ornithine or modified ornithine wherein the modified ornithine is an ornithine forming an amide bond with a linker through the d-amino group
  MOD_RES 6: Native ornithine or modified ornithine wherein the modified ornithine is an ornithine forming an amide bond with a linker through the d-amino group
  MOD_RES 7: AMIDATION
RXHRXXH

SEQ ID NO: 53 - protein, 7 aa, Artificial Sequence
  MOD_RES 1: ACETYLATION
  Cationic peptide R + 7.3(L-H)-H
  MOD_RES 3: Native lysine or modified lysine, wherein the modified lysine is a lysine forming an amide bond with a linker through the e-amino group.
  MOD_RES 6: Native lysine or modified lysine, wherein the modified lysine is a lysine forming an amide bond with a linker through the e-amino group
  MOD_RES 7: Native lysine or modified lysine wherein the modified lysine is a lysine forming an amide bond with a linker through the e-amino group
  MOD_RES 7: AMIDATION
RRKHRKK

SEQ ID NO: 54 - protein, 8 aa, Artificial Sequence
  MOD_RES 1: ACETYLATION
  Cationic peptide R + 7.3(L-H)
  MOD_RES 3: Native lysine or modified lysine, wherein the modified lysine is a lysine forming an amide bond with a linker through the e-amino group
  MOD_RES 6: Native lysine or modified lysine, wherein the modified lysine is a lysine forming an amide bond with a linker through the e-amino group
  MOD_RES 7: Native lysine or modified lysine, wherein the modified lysine is a lysine forming an amide bond with a linker through the e-amino group
  MOD_RES 8: AMIDATION
RRKHRKKH

SEQ ID NO: 55 - protein, 7 aa, Artificial Sequence
  MOD_RES 1: ACETYLATION
  Cationic peptide R + 7.3-Â L
  MOD_RES 3: Native lysine or modified lysine, wherein the modified lysine is a lysine forming an amide bond with a linker through the e-amino group
  MOD_RES 6: Native lysine or modified lysine, wherein the modified lysine is a lysine forming an amide bond with a linker through the e-amino group
  MOD_RES 7: Native lysine or modified lysine, wherein the modified lysine is a lysine forming an amide bond with a linker through the e-amino group
  MOD_RES 7: AMIDATION
RRKLRKK

SEQ ID NO: 56 - protein, 8 aa, Artificial Sequence
  MOD_RES 1: ACETYLATION
  Cationic peptide R + 7.3
  MOD_RES 3: Native lysine or modified lysine, wherein the modified lysine is a lysine forming an amide bond with a linker through the e-amino group
  MOD_RES 6: Native lysine or modified lysine, wherein the modified lysine is a lysine forming an amide bond with a linker through the e-amino group
  MOD_RES 7: Native lysine or modified lysine, wherein the modified lysine is a lysine forming an amide bond with a linker through the e-amino group
  MOD_RES 8: AMIDATION
RRKLRKKL

SEQ ID NO: 57 - protein, 9 aa, Artificial Sequence
  MOD_RES 1: ACETYLATION
  Cationic peptide RR + 7.3
  MOD_RES 4: Native lysine or modified lysine, wherein the modified lysine is a lysine forming an amide bond with a linker through the e-amino group
  MOD_RES 7: Native lysine or modified lysine, wherein the modified lysine is a lysine forming an amide bond with a linker through the e-amino group
  MOD_RES 8: Native lysine or modified lysine, wherein the modified lysine is a lysine forming an amide bond with a linker through the e-amino group
  MOD_RES 9: AMIDATION
RRRKLRKKL

SEQ ID NO: 58 - protein, 7 aa, Artificial Sequence
  MOD_RES 1: ACETYLATION
  Cationic peptide V3-7.3(L-H)
  MOD_RES 2: Native ornithine or modified ornithine wherein the modified ornithine is an ornithine forming an amide bond with a linker through the d-amino group
  MOD_RES 5: Native lysine or modified lysine, wherein the modified lysine is a lysine forming an amide bond with a linker through the e-amino group
  MOD_RES 6: Native lysine or modified lysine, wherein the modified lysine is a lysine forming an amide bond with a linker through the e-amino group
  MOD_RES 7: AMIDATION
RXHRKKH

SEQ ID NO: 59 - protein, 7 aa, Artificial Sequence
  MOD_RES 1: ACETYLATION
  Cationic peptide V4-7.3(L-H)
  MOD_RES 2: Native lysine or modified lysine, wherein the modified lysine is a lysine forming an amide bond with a linker through the e-amino group
  MOD_RES 5: Native lysine or modified lysine, wherein the modified lysine is a lysine forming an amide bond with a linker through the e-amino group
  MOD_RES 6: Native ornithine or modified ornithine wherein the modified ornithine is an ornithine forming an amide bond with a linker through the d-amino group
  MOD_RES 7: AMIDATION
RKHRKXH

SEQ ID NO: 60 - DNA, 22 bp, Artificial Sequence
  TLR9 agonist CpG (ODN2395)
  modified_base 1..22: /mod_base="OTHER" /note="bases are phosphorothioates"
tcgtcgttttcggcgcgcgccg

SEQ ID NO: 61 - RNA, 1653 nt, Artificial Sequence
  mRNA sequence encoding the firefly luciferase protein - CleanCap FLuc mRNA Open Reading Frame Sequence
auggaggacgccaagaacaucaagaagggccccgcccccuucuacccccuggaggacggcaccgccggcgagcagcugcacaaggccaugaagcgguacgcccuggugcccggcaccaucgccuucaccgacgcccacaucgagguggacaucaccuacgccgaguacuucgagaugagcgugcggcuggccgaggccaugaagcgguacggccugaacaccaaccaccggaucguggugugcagcgagaacagccugcaguucuucaugcccgugcugggcgcccuguucaucggcguggccguggcccccgccaacgacaucuacaacgagcgggagcugcugaacagcaugggcaucagccagcccaccgugguguucgugagcaagaagggccugcagaagauccugaacgugcagaagaagcugcccaucauccagaagaucaucaucauggacagcaagaccgacuaccagggcuuccagagcauguacaccuucgugaccagccaccugccccccggcuucaacgaguacgacuucgugcccgagagcuucgaccgggacaagaccaucgcccugaucaugaacagcagcggcagcaccggccugcccaagggcguggcccugccccaccggaccgccugcgugcgguucagccacgcccgggaccccaucuucggcaaccagaucauccccgacaccgccauccugagcguggugcccuuccaccacggcuucggcauguucaccacccugggcuaccugaucugcggcuuccggguggugcugauguaccgguucgaggaggagcuguuccugcggagccugcaggacuacaagauccagagcgcccugcuggugcccacccuguucagcuucuucgccaagagcacccugaucgacaaguacgaccugagcaaccugcacgagaucgccagcggcggcgccccccugagcaaggaggugggcgaggccguggccaagcgguuccaccugcccggcauccggcagggcuacggccugaccgagaccaccagcgccauccugaucacccccgagggcgacgacaagcccggcgccgugggcaagguggugcccuucuucgaggccaaggugguggaccuggacaccggcaagacccugggcgugaaccagcggggcgagcugugcgugcggggccccaugaucaugagcggcuacgugaacaaccccgaggccaccaacgcccugaucgacaaggacggcuggcugcacagcggcgacaucgccuacugggacgaggacgagcacuucuucaucguggaccggcugaagagccugaucaaguacaagggcuaccagguggcccccgccgagcuggagagcauccugcugcagcaccccaacaucuucgacgccggcguggccggccugcccgacgacgacgccggcgagcugcccgccgccgugguggugcuggagcacggcaagaccaugaccgagaaggagaucguggacuacguggccagccaggugaccaccgccaagaagcugcggggcggcgugguguucguggacgaggugcccaagggccugaccggcaagcuggacgcccggaagauccgggagauccugaucaaggccaagaagggcggcaagaucgccguguga

SEQ ID NO: 62 - RNA, 720 nt, Artificial Sequence
  CleanCap EGFP mRNA Open Reading Frame Sequence
auggugagcaagggcgaggagcuguucaccgggguggugcccauccuggucgagcuggacggcgacguaaacggccacaaguucagcguguccggcgagggcgagggcgaugccaccuacggcaagcugacccugaaguucaucugcaccaccggcaagcugcccgugcccuggcccacccucgugaccacccugaccuacggcgugcagugcuucagccgcuaccccgaccacaugaagcagcacgacuucuucaaguccgccaugcccgaaggcuacguccaggagcgcaccaucuucuucaaggacgacggcaacuacaagacccgcgccgaggugaaguucgagggcgacacccuggugaaccgcaucgagcugaagggcaucgacuucaaggaggacggcaacauccuggggcacaagcuggaguacaacuacaacagccacaacgucuauaucauggccgacaagcagaagaacggcaucaaggugaacuucaagauccgccacaacaucgaggacggcagcgugcagcucgccgaccacuaccagcagaacacccccaucggcgacggccccgugcugcugcccgacaaccacuaccugagcacccaguccgcccugagcaaagaccccaacgagaagcgcgaucacaugguccugcuggaguucgugaccgccgccgggaucacucucggcauggacgagcuguacaaguaa

SEQ ID NO: 63 - RNA, 1161 nt, Artificial Sequence
  CleanCap OVA mRNA Open Reading Frame Sequence
augggcagcaucggcgccgccagcauggaguucugcuucgacguguucaaggagcugaaggugcaccacgccaacgagaacaucuucuacugccccaucgccaucaugagcgcccuggccaugguguaccugggcgccaaggacagcacccggacccagaucaacaagguggugcgguucgacaagcugcccggcuucggcgacagcaucgaggcccagugcggcaccagcgugaacgugcacagcagccugcgggacauccugaaccagaucaccaagcccaacgacguguacagcuucagccuggccagccggcuguacgccgaggagcgguaccccauccugcccgaguaccugcagugcgugaaggagcuguaccggggcggccuggagcccaucaacuuccagaccgccgccgaccaggcccgggagcugaucaacagcuggguggagagccagaccaacggcaucauccggaacgugcugcagcccagcagcguggacagccagaccgccauggugcuggugaacgccaucguguucaagggccugugggagaagaccuucaaggacgaggacacccaggccaugcccuuccgggugaccgagcaggagagcaagcccgugcagaugauguaccagaucggccuguuccggguggccagcauggccagcgagaagaugaagauccuggagcugcccuucgccagcggcaccaugagcaugcuggugcugcugcccgacgaggugagcggccuggagcagcuggagagcaucaucaacuucgagaagcugaccgaguggaccagcagcaacgugauggaggagcggaagaucaagguguaccugccccggaugaagauggaggagaaguacaaccugaccagcgugcugauggccaugggcaucaccgacguguucagcagcagcgccaaccugagcggcaucagcagcgccgagagccugaagaucagccaggccgugcacgccgcccacgccgagaucaacgaggccggccgggagguggugggcagcgccgaggccggcguggacgccgccagcgugagcgaggaguuccgggccgaccaccccuuccuguucugcaucaagcacaucgccaccaacgccgugcuguucuucggccggugcgugagccccuga

SEQ ID NO: 64 - protein, 8 aa, Artificial Sequence
  Immunogenic fragment from OVA
SIINFEKL